European Patent Specification EP 3 560 953 B1, published January 31, 2024. Title: CELL. Applicant: UCL Business PLC Autolus Ltd. The sequence listing filed with the application follows.

SEQUENCE LISTING (49 sequences)

SEQ ID NO: 1 - protein, 21 aa, Artificial Sequence
  Signal peptide
MGTSLLCWMALCLLGADHADG

SEQ ID NO: 2 - protein, 21 aa, Artificial Sequence
  Signal peptide
MSLPVTALLLPLALLLHAARP

SEQ ID NO: 3 - protein, 20 aa, Artificial Sequence
  Signal peptide
MAVPTQVLGLLLLWLTDARC

SEQ ID NO: 4 - protein, 234 aa, Artificial Sequence
  spacer sequence, hinge-CH2CH3 of human IgG1
AEPKSPDKTHTCPPCPAPPVAGPSVFLFPPKPKDTLMIARTPEVTCVVVDVSHEDPEVKFNWYVDGVEVHNAKTKPREEQYNSTYRVVSVLTVLHQDWLNGKEYKCKVSNKALPAPIEKTISKAKGQPREPQVYTLPPSRDELTKNQVSLTCLVKGFYPSDIAVEWESNGQPENNYKTTPPVLDSDGSFFLYSKLTVDKSRWQQGNVFSCSVMHEALHNHYTQKSLSLSPGKKD

SEQ ID NO: 5 - protein, 46 aa, Artificial Sequence
  spacer sequence, human CD8 stalk
TTTPAPRPPTPAPTIASQPLSLRPEACRPAAGGAVHTRGLDFACDI

SEQ ID NO: 6 - protein, 20 aa, Artificial Sequence
  spacer sequence, human IgG1 hinge
AEPKSPDKTHTCPPCPKDPK

SEQ ID NO: 7 - protein, 185 aa, Artificial Sequence
  spacer sequence, CD2 ectodomain
KEITNALETWGALGQDINLDIPSFQMSDDIDDIKWEKTSDKKKIAQFRKEKETFKEKDTYKLFKNGTLKIKHLKTDDQDIYKVSIYDTKGKNVLEKIFDLKIQERVSKPKISWTCINTTLTCEVMNGTDPELNLYQDGKHLKLSQRVITHKWTTSLSAKFKCTAGNKVSKESSVEPVSCPEKGLD

SEQ ID NO: 8 - protein, 259 aa, Artificial Sequence
  spacer sequence, CD34 ectodomain
SLDNNGTATPELPTQGTFSNVSTNVSYQETTTPSTLGSTSLHPVSQHGNEATTNITETTVKFTSTSVITSVYGNTNSSVQSQTSVISTVFTTPANVSTPETTLKPSLSPGNVSDLSTTSTSLATSPTKPYTSSSPILSDIKAEIKCSGIREVKLTQGICLEQNKTSSCAEFKKDRGEGLARVLCGEEQADADAGAQVCSLLLAQSEVRPQCLLLVLANRTEISSKLQLMKKHQSDLKKLGILDFTEQDVASHQSYSQKT

SEQ ID NO: 9 - protein, 140 aa, Artificial Sequence
  comprising CD28 transmembrane domain and CD3 Z endodomain
FWVLVVVGGVLACYSLLVTVAFIIFWVRRVKFSRSADAPAYQQGQNQLYNELNLGRREEYDVLDKRRGRDPEMGGKPRRKNPQEGLYNELQKDKMAEAYSEIGMKGERRRGKGHDGLYQGLSTATKDTYDALHMQALPPR

SEQ ID NO: 10 - protein, 180 aa, Artificial Sequence
  comprising CD28 transmembrane domain and CD28 and CD3 Zeta endodomains
FWVLVVVGGVLACYSLLVTVAFIIFWVRSKRSRLLHSDYMNMTPRRPGPTRKHYQPYAPPRDFAAYRSRVKFSRSADAPAYQQGQNQLYNELNLGRREEYDVLDKRRGRDPEMGGKPRRKNPQEGLYNELQKDKMAEAYSEIGMKGERRRGKGHDGLYQGLSTATKDTYDALHMQALPPR

SEQ ID NO: 11 - protein, 216 aa, Artificial Sequence
  comprising CD28 transmembrane domain and CD28, OX40 and CD3 Zeta endodomains
FWVLVVVGGVLACYSLLVTVAFIIFWVRSKRSRLLHSDYMNMTPRRPGPTRKHYQPYAPPRDFAAYRSRDQRLPPDAHKPPGGGSFRTPIQEEQADAHSTLAKIRVKFSRSADAPAYQQGQNQLYNELNLGRREEYDVLDKRRGRDPEMGGKPRRKNPQEGLYNELQKDKMAEAYSEIGMKGERRRGKGHDGLYQGLSTATKDTYDALHMQALPPR

SEQ ID NO: 12 - protein, 20 aa, Artificial Sequence
  2A-like sequence
RAEGRGSLLTCGDVEENPGP

SEQ ID NO: 13 - DNA, 3402 bp, Artificial Sequence
  CD19/CD22 'OR' gate construct
atgagcctgcccgtgaccgccctgctgctgcccctggccctgctgctgcacgccgccagaccatacccctacgacgtgcccgactacgccagcctgagcggaggcggcggcagccaggtgcagctggtgcagagcggagccgaggtgaagaagcctggcgccagcgtgaaggtgtcctgtaaggccagcggctacaccttcaccagcaactggatgcactgggtgaggcaggcccctggacagggactggagtggatgggcgagatcgaccccagcgacagctacaccaactacaaccagaagttcaagggccgggtgaccatcaccgtggataagagcgccagcaccgcctacatggagctgtccagcctgagaagcgaggataccgccgtgtactactgtgccagaggcagcaacccctactactacgctatggactactggggccagggcaccctggtgaccgtgtccagcggcggaggaggaagcggagggggcggatctggcggcggagggagcgagatcgtgctgacccagagccccgccaccctgagcctgagccctggcgagagagccaccctgtcctgtagcgccagcagcggcgtgaattacatgcactggtatcagcagaagcccggccaggcccccagaagatggatctacgacaccagcaagctggccagcggcgtgcccgccagattcagcggcagcggctccggcaccagctacagcctgaccatcagcagcctggagcctgaggatttcgccgtgtattattgccaccagaggggcagctacacctttggcggcggaacaaagctggagatcaagcgctcagatcccaccacgacgccagcgccgcgaccaccaacaccggcgcccaccatcgcgtcgcagcccctgtccctgcgcccagaggcgtgccggccagcggcggggggcgcagtgcacacgagggggctggacttcgcctgtgatatcttttgggtgctggtggtggttggtggagtcctggcttgctatagcttgctagtaacagtggcctttattattttctgggtgaggagagtgaagttcagcaggagcgcagacgcccccgcgtaccagcagggccagaaccagctctataacgagctcaatctaggacgaagagaggagtacgatgttttggacaagagacgtggccgggaccctgagatggggggaaagccgagaaggaagaaccctcaggaaggcctgtacaatgaactgcagaaagataagatggcggaggcctacagtgagattgggatgaaaggcgagcgccggaggggcaaggggcacgatggcctttaccagggtctcagtacagccaccaaggacacctacgacgcccttcacatgcaggccctgcctcctcgcagagccgagggcaggggaagtcttctaacatgcggggacgtggaggaaaatcccgggcccatggagtttgggctgagctggctttttcttgtggctattttaaaaggtgtccagtgcgaggtgcagctggtggagtctgggggaggcttggtccagccaggggggtccctgcgcctctcctgtgcagcctctggattcgctttcagtatctatgacatgtcttgggtccgccaggttccggggaaggggctggagtgggtctcatatattagtagtggtggtggtaccacctattacccggacactgtgaagggccgcttcaccatctcccgtgacaattcccgcaacactctggatcttcaaatgaacagtctgcgcgtcgaggacacggctgtctattattgtgcgcgtcatagtggctacggtagtagctacggggttttgtttgcttactggggccaaggaaccctggtcaccgtctcctcaggtggaggcggttcaggcggaggtggctctggcggtggcggatcggacatccagatgactcagtctccgtcctccctgtctgcatctgtaggagaccgcgtcaccatcacctgccgtgcaagtcaggacattagcaattatttaaactggcttcaacagaaaccggggaaagccccgaagctcctgatttactacacatcaatcttacactcaggagtcccgtcacgcttcagcggcagtggatctgggacagaattcactctcacaatcagcagcctgcagccggaagattttgcaacttattactgtcaacagggtaatacgcttccgtggacgtttggccaggggaccaaactggaaatcaaacgttcggatccagccgaaccaaagagccccgataagacccacacctgtcccccctgcccagccccagagctgctgggaggccccagcgtgtttctgtttccacccaagccaaaggataccctgatgattagtagaacacccgaagtgacctgtgtggtggtggatgtgtctcacgaggaccccgaggtgaaatttaattggtatgttgatggtgttgaagtgcacaacgccaaaaccaaacccagagaggagcagtacaattctacctatagagtcgtgtctgtgctgacagtgctgcatcaggattggctgaacggaaaagaatacaaatgtaaagtgagcaataaggccctgcccgctccaattgagaagacaattagcaaggccaagggccagccaagggagccccaggtgtatacactgccacccagtagagacgaactgacaaagaatcaggtgtctctgacatgtctggtgaagggattttacccatctgatatcgccgtggaatgggaatctaacggccagcccgagaataactataagacaaccccaccagtgctggatagcgatggcagcttttttctgtattctaagctgacagtggataagtcccggtggcagcagggaaatgtgtttagctgtagtgtcatgcatgaggccctgcacaatcactatacccagaaatctctgagtctgagcccaggcaagaaggaccccaagttctgggtcctggtggtggtgggaggcgtgctggcctgttactctctcctggtgaccgtggccttcatcatcttttgggtgcgctcccgggtgaagttttctcgctctgccgatgccccagcctatcagcagggccagaatcagctgtacaatgaactgaacctgggcaggcgggaggagtacgacgtgctggataagcggagaggcagagaccccgagatgggcggcaaaccacggcgcaaaaatccccaggagggactctataacgagctgcagaaggacaaaatggccgaggcctattccgagatcggcatgaagggagagagaagacgcggaaagggccacgacggcctgtatcagggattgtccaccgctacaaaagatacatatgatgccctgcacatgcaggccctgccacccagatga

SEQ ID NO: 14 - protein, 1133 aa, Artificial Sequence
  CD19/CD22 'OR' gate construct
MSLPVTALLLPLALLLHAARPYPYDVPDYASLSGGGGSQVQLVQSGAEVKKPGASVKVSCKASGYTFTSNWMHWVRQAPGQGLEWMGEIDPSDSYTNYNQKFKGRVTITVDKSASTAYMELSSLRSEDTAVYYCARGSNPYYYAMDYWGQGTLVTVSSGGGGSGGGGSGGGGSEIVLTQSPATLSLSPGERATLSCSASSGVNYMHWYQQKPGQAPRRWIYDTSKLASGVPARFSGSGSGTSYSLTISSLEPEDFAVYYCHQRGSYTFGGGTKLEIKRSDPTTTPAPRPPTPAPTIASQPLSLRPEACRPAAGGAVHTRGLDFACDIFWVLVVVGGVLACYSLLVTVAFIIFWVRRVKFSRSADAPAYQQGQNQLYNELNLGRREEYDVLDKRRGRDPEMGGKPRRKNPQEGLYNELQKDKMAEAYSEIGMKGERRRGKGHDGLYQGLSTATKDTYDALHMQALPPRRAEGRGSLLTCGDVEENPGPMEFGLSWLFLVAILKGVQCEVQLVESGGGLVQPGGSLRLSCAASGFAFSIYDMSWVRQVPGKGLEWVSYISSGGGTTYYPDTVKGRFTISRDNSRNTLDLQMNSLRVEDTAVYYCARHSGYGSSYGVLFAYWGQGTLVTVSSGGGGSGGGGSGGGGSDIQMTQSPSSLSASVGDRVTITCRASQDISNYLNWLQQKPGKAPKLLIYYTSILHSGVPSRFSGSGSGTEFTLTISSLQPEDFATYYCQQGNTLPWTFGQGTKLEIKRSDPAEPKSPDKTHTCPPCPAPELLGGPSVFLFPPKPKDTLMISRTPEVTCVVVDVSHEDPEVKFNWYVDGVEVHNAKTKPREEQYNSTYRVVSVLTVLHQDWLNGKEYKCKVSNKALPAPIEKTISKAKGQPREPQVYTLPPSRDELTKNQVSLTCLVKGFYPSDIAVEWESNGQPENNYKTTPPVLDSDGSFFLYSKLTVDKSRWQQGNVFSCSVMHEALHNHYTQKSLSLSPGKKDPKFWVLVVVGGVLACYSLLVTVAFIIFWVRSRVKFSRSADAPAYQQGQNQLYNELNLGRREEYDVLDKRRGRDPEMGGKPRRKNPQEGLYNELQKDKMAEAYSEIGMKGERRRGKGHDGLYQGLSTATKDTYDALHMQALPPR

SEQ ID NO: 15 - protein, 5 aa, Artificial Sequence
  Complementarity determining region (CDR) variable heavy chain (VH) CDR1
SYWMN

SEQ ID NO: 16 - protein, 16 aa, Artificial Sequence
  VH CDR2
QIWPGDGDTNYNGKFK

SEQ ID NO: 17 - protein, 15 aa, Artificial Sequence
  VH CDR3
RETTTVGRYYYAMDY

SEQ ID NO: 18 - protein, 15 aa, Artificial Sequence
  Variable light chain (VL) CDR1
KASQSVDYDGDSYLN

SEQ ID NO: 19 - protein, 7 aa, Artificial Sequence
  VL CDR2
DASNLVS

SEQ ID NO: 20 - protein, 9 aa, Artificial Sequence
  VL CDR3
QQSTEDPWT

SEQ ID NO: 21 - protein, 235 aa, Artificial Sequence
  chimeric antigen receptor (CAR), Murine CD19ALAb scFv sequence
QVQLQQSGAELVRPGSSVKISCKASGYAFSSYWMNWVKQRPGQGLEWIGQIWPGDGDTNYNGKFKGKATLTADESSSTAYMQLSSLASEDSAVYFCARRETTTVGRYYYAMDYWGQGTTVTVSSDIQLTQSPASLAVSLGQRATISCKASQSVDYDGDSYLNWYQQIPGQPPKLLIYDASNLVSGIPPRFSGSGSGTDFTLNIHPVEKVDAATYHCQQSTEDPWTFGGGTKLEIK

SEQ ID NO: 22 - protein, 236 aa, Artificial Sequence
  CAR, Humanised CD19ALAb scFv sequence - Heavy 19, Kappa 16
QVQLVQSGAEVKKPGASVKLSCKASGYAFSSYWMNWVRQAPGQSLEWIGQIWPGDGDTNYNGKFKGRATLTADESARTAYMELSSLRSGDTAVYFCARRETTTVGRYYYAMDYWGKGTLVTVSSDIQLTQSPDSLAVSLGERATINCKASQSVDYDGDSYLNWYQQKPGQPPKLLIYDASNLVSGVPDRFSGSGSGTDFTLTISSLQAADVAVYHCQQSTEDPWTFGQGTKVEIKR

SEQ ID NO: 23 - protein, 124 aa, Artificial Sequence
  CAR, Murine CD19ALAb VH sequence
QVQLQQSGAELVRPGSSVKISCKASGYAFSSYWMNWVKQRPGQGLEWIGQIWPGDGDTNYNGKFKGKATLTADESSSTAYMQLSSLASEDSAVYFCARRETTTVGRYYYAMDYWGQGTTVTVSS

SEQ ID NO: 24 - protein, 124 aa, Artificial Sequence
  CAR, Humanised CD19ALAb VH sequence
QVQLVQSGAEVKKPGASVKLSCKASGYAFSSYWMNWVRQAPGQSLEWIGQIWPGDGDTNYNGKFKGRATLTADESARTAYMELSSLRSGDTAVYFCARRETTTVGRYYYAMDYWGKGTLVTVSS

SEQ ID NO: 25 - protein, 111 aa, Artificial Sequence
  CAR, Murine CD19ALAb VL sequence
DIQLTQSPASLAVSLGQRATISCKASQSVDYDGDSYLNWYQQIPGQPPKLLIYDASNLVSGIPPRFSGSGSGTDFTLNIHPVEKVDAATYHCQQSTEDPWTFGGGTKLEIK

SEQ ID NO: 26 - protein, 112 aa, Artificial Sequence
  CAR, Humanised CD19ALAb VL sequence, Kappa16
DIQLTQSPDSLAVSLGERATINCKASQSVDYDGDSYLNWYQQKPGQPPKLLIYDASNLVSGVPDRFSGSGSGTDFTLTISSLQAADVAVYHCQQSTEDPWTFGQGTKVEIKR

SEQ ID NO: 27 - protein, 5 aa, Artificial Sequence
  VH CDR1
NYWIN

SEQ ID NO: 28 - protein, 17 aa, Artificial Sequence
  VH CDR2
NIYPSDSFTNYNQKFKD

SEQ ID NO: 29 - protein, 11 aa, Artificial Sequence
  VH CDR3
DTQERSWYFDV

SEQ ID NO: 30 - protein, 16 aa, Artificial Sequence
  VL CDR1
RSSQSLVHSNGNTYLH

SEQ ID NO: 31 - protein, 7 aa, Artificial Sequence
  VL CDR2
KVSNRFS

SEQ ID NO: 32 - protein, 9 aa, Artificial Sequence
  VL CDR3
SQSTHVPWT

SEQ ID NO: 33 - protein, 232 aa, Artificial Sequence
  CAR, Murine CD22ALAb scFv sequence
QVQLQQPGAELVRPGASVKLSCKASGYTFTNYWINWVKQRPGQGLEWIGNIYPSDSFTNYNQKFKDKATLTVDKSSSTAYMQLSSPTSEDSAVYYCTRDTQERSWYFDVWGAGTTVTVSSDVVMTQTPLSLPVSLGDQASISCRSSQSLVHSNGNTYLHWYLQKPGQSPKLLIYKVSNRFSGVPDRFSGSGSGTDFTLKISRVEAEDLGLYFCSQSTHVPWTFGGGTKLEIK

SEQ ID NO: 34 - protein, 232 aa, Artificial Sequence
  CAR, Humanised CD22ALAb scFv sequence
EVQLVESGAEVKKPGSSVKVSCKASGYTFTNYWINWVRQAPGQGLEWIGNIYPSDSFTNYNQKFKDRATLTVDKSTSTAYLELRNLRSDDTAVYYCTRDTQERSWYFDVWGQGTLVTVSSDIVMTQSPATLSVSPGERATLSCRSSQSLVHSNGNTYLHWYQQKPGQAPRLLIYKVSNRFSGVPARFSGSGSGVEFTLTISSLQSEDFAVYYCSQSTHVPWTFGQGTRLEIK

SEQ ID NO: 35 - protein, 120 aa, Artificial Sequence
  CAR, Murine CD22ALAb VH sequence
QVQLQQPGAELVRPGASVKLSCKASGYTFTNYWINWVKQRPGQGLEWIGNIYPSDSFTNYNQKFKDKATLTVDKSSSTAYMQLSSPTSEDSAVYYCTRDTQERSWYFDVWGAGTTVTVSS

SEQ ID NO: 36 - protein, 120 aa, Artificial Sequence
  CAR, Humanised CD22ALAb VH sequence
EVQLVESGAEVKKPGSSVKVSCKASGYTFTNYWINWVRQAPGQGLEWIGNIYPSDSFTNYNQKFKDRATLTVDKSTSTAYLELRNLRSDDTAVYYCTRDTQERSWYFDVWGQGTLVTVSS

SEQ ID NO: 37 - protein, 112 aa, Artificial Sequence
  CAR, Murine CD22ALAb VL sequence
DVVMTQTPLSLPVSLGDQASISCRSSQSLVHSNGNTYLHWYLQKPGQSPKLLIYKVSNRFSGVPDRFSGSGSGTDFTLKISRVEAEDLGLYFCSQSTHVPWTFGGGTKLEIK

SEQ ID NO: 38 - protein, 112 aa, Artificial Sequence
  CAR, Humanised CD22ALAb VL sequence
DIVMTQSPATLSVSPGERATLSCRSSQSLVHSNGNTYLHWYQQKPGQAPRLLIYKVSNRFSGVPARFSGSGSGVEFTLTISSLQSEDFAVYYCSQSTHVPWTFGQGTRLEIK

SEQ ID NO: 39 - protein, 236 aa, Artificial Sequence
  CAR, Humanised CD19ALAb scFv sequence - Heavy 19, Kappa 7
QVQLVQSGAEVKKPGASVKLSCKASGYAFSSYWMNWVRQAPGQSLEWIGQIWPGDGDTNYNGKFKGRATLTADESARTAYMELSSLRSGDTAVYFCARRETTTVGRYYYAMDYWGKGTLVTVSSDIQLTQSPDSLAVSLGERATINCKASQSVDYDGDSYLNWYQQKPGQPPKVLIYDASNLVSGVPDRFSGSGSGTDFTLTISSLQAADVAVYYCQQSTEDPWTFGQGTKVEIKR

SEQ ID NO: 40 - protein, 112 aa, Artificial Sequence
  CAR, Humanised CD19ALAb VL sequence, Kappa 7
DIQLTQSPDSLAVSLGERATINCKASQSVDYDGDSYLNWYQQKPGQPPKVLIYDASNLVSGVPDRFSGSGSGTDFTLTISSLQAADVAVYYCQQSTEDPWTFGQGTKVEIKR

SEQ ID NO: 41 - protein, 40 aa, Artificial Sequence
  CD28 co-stimulatory endodomain
SKRSRLLHSDYMNMTPRRPGPTRKHYQPYAPPRDFAAYRS

SEQ ID NO: 42 - protein, 36 aa, Artificial Sequence
  OX40 endodomain
RDQRLPPDAHKPPGGGSFRTPIQEEQADAHSTLAKI

SEQ ID NO: 43 - protein, 42 aa, Artificial Sequence
  4-1BB endodomain
KRGRKKLLYIFKQPFMRPVQTTQEEDGCSCRFPEEEEGGCEL

SEQ ID NO: 44 - protein, 112 aa, Artificial Sequence
  CD3zeta endodomain
RVKFSRSADAPAYQQGQNQLYNELNLGRREEYDVLDKRRGRDPEMGGKPRRKNPQEGLYNELQKDKMAEAYSEIGMKGERRRGKGHDGLYQGLSTATKDTYDALHMQALPPR

SEQ ID NO: 45 - protein, 24 aa, Artificial Sequence
  Tyrp-1 transmembrane sequence
IIAIAVVGALLLVALIFGTASYLI

SEQ ID NO: 46 - protein, 258 aa, Homo sapiens
EEPLVVKVEEGDNAVLQCLKGTSDGPTQQLTWSRESPLKPFLKLSLGLPGLGIHMRPLAIWLFIFNVSQQMGGFYLCQPGPPSEKAWQPGWTVNVEGSGELFRWNVSDLGGLGCGLKNRSSEGPSSPSGKLMSPKLYVWAKDRPEIWEGEPPCLPPRDSLNQSLSQDLTMAPGSTLWLSCGVPPDSVSRGPLSWTHVHPKGPKSLLSLELKDDRPARDMWVMETGLLLPRATAQDAGKYYCHRGNLTMSFHLEITARP

SEQ ID NO: 47 - protein, 4 aa, Artificial Sequence
  ITAM motif
  misc_feature (2)..(3): Xaa can be any naturally occurring amino acid
  MISC_FEATURE (4)..(4): Xaa may be leucine or isoleucine
YXXX

SEQ ID NO: 48 - DNA, 1139 bp, Homo sapiens
atcccgccgagcccaaatctcctgacaaaactcacacatgcccaccgtgcccagcacctgaactcctggggggaccgtcagtcttcctcttccccccaaaacccaaggacaccctcatgatctcccggacccctgaggtcacatgcgtggtggtggacgtgagccacgaagaccctgaggtcaagttcaactggtacgtggacggcgtggaggtgcataatgccaagacaaagccgcgggaggagcagtacaacagcacgtaccgtgtggtcagcgtcctcaccgtcctgcaccaggactggctgaatggcaaggagtacaagtgcaaggtctccaacaaagccctcccagcccccatcgagaaaaccatctccaaagccaaagggcagccccgagaaccacaggtgtacaccctgcccccatcccgggatgagctgaccaagaaccaggtcagcctgacctgcctggtcaaaggcttctatcccagcgacatcgccgtggagtgggagagcaatgggcaaccggagaacaactacaagaccacgcctcccgtgctggactccgacggctccttcttcctctacagcaagctcaccgtggacaagagcaggtggcagcaggggaacgtcttctcatgctccgtgatgcacgaggctctgcacaaccactacacgcagaagagcctctccctgtctccgggtaaaaaagatcccaaattttgggtgctggtggtggttggtggagtcctggcttgctatagcttgctagtaacagtggcctttattattttctgggtgaggagagtgaagttcagcaggagcgcagacgcccccgcgtaccagcagggccagaaccagctctataacgagctcaatctaggacgaagagaggagtacgatgttttggacaagagacgtggccgggaccctgagatggggggaaagccgagaaggaagaaccctcaggaaggcctgtacaatgaactgcagaaagataagatggcggaggcctacagtgagattgggatgaaaggcgagcgccggaggggcaaggggcacgatggcctttaccagggtctcagtacagccaccaaggacacctacgacgcccttcacatgcaggccctgcctcctcgcgag

SEQ ID NO: 49 - DNA, 1139 bp, Artificial Sequence
  codon-wobbled HCH2CH3-CD28tmZeta
atccagccgaaccaaagagccccgataagacccacacctgtcccccctgcccagccccagagctgctgggaggccccagcgtgtttctgtttccacccaagccaaaggataccctgatgattagtagaacacccgaagtgacctgtgtggtggtggatgtgtctcacgaggaccccgaggtgaaatttaattggtatgttgatggtgttgaagtgcacaacgccaaaaccaaacccagagaggagcagtacaattctacctatagagtcgtgtctgtgctgacagtgctgcatcaggattggctgaacggaaaagaatacaaatgtaaagtgagcaataaggccctgcccgctccaattgagaagacaattagcaaggccaagggccagccaagggagccccaggtgtatacactgccacccagtagagacgaactgacaaagaatcaggtgtctctgacatgtctggtgaagggattttacccatctgatatcgccgtggaatgggaatctaacggccagcccgagaataactataagacaaccccaccagtgctggatagcgatggcagcttttttctgtattctaagctgacagtggataagtcccggtggcagcagggaaatgtgtttagctgtagtgtcatgcatgaggccctgcacaatcactatacccagaaatctctgagtctgagcccaggcaagaaggaccccaagttctgggtcctggtggtggtgggaggcgtgctggcctgttactctctcctggtgaccgtggccttcatcatcttttgggtgcgctcccgggtgaagttttctcgctctgccgatgccccagcctatcagcagggccagaatcagctgtacaatgaactgaacctgggcaggcgggaggagtacgacgtgctggataagcggagaggcagagaccccgagatgggcggcaaaccacggcgcaaaaatccccaggagggactctataacgagctgcagaaggacaaaatggccgaggcctattccgagatcggcatgaagggagagagaagacgcggaaagggccacgacggcctgtatcagggattgtccaccgctacaaaagatacatatgatgccctgcacatgcaggccctgccacccaga